European Patent Application EP 4 279 505 A1, published November 22, 2023. Title: HUMAN CD276-TARGETING MONOCLONAL ANTIBODY AND APPLICATION THEREOF. Applicant: PERSONGEN BIOTHERAPEUTICS (SUZHOU) CO., LTD. The sequence listing filed with the application follows.

SEQUENCE LISTING (33 sequences)

SEQ ID NO: 1 - protein, 7 aa, Mus musculus
GFTFSTY

SEQ ID NO: 2 - protein, 5 aa, Mus musculus
LSGGT

SEQ ID NO: 3 - protein, 12 aa, Mus musculus
RYGHDHYYAMDY

SEQ ID NO: 4 - protein, 12 aa, Mus musculus
AASSSVSSSYLH

SEQ ID NO: 5 - protein, 7 aa, Mus musculus
STSNLAS

SEQ ID NO: 6 - protein, 8 aa, Mus musculus
QYHRSPWT

SEQ ID NO: 7 - protein, 12 aa, Mus musculus
RYGHDRYYAMDY

SEQ ID NO: 8 - protein, 120 aa, Mus musculus
EVTLVESGGGLVKPGGSLKLSCAASGFTFSTYVMSWVRQTPEKRLEWVASILSGGTSFYADNVKGRFTISRENARNILYLQMSSLKSEDTAMYYCVRRYGHDRYYAMDYWGQGTSVTVSS

SEQ ID NO: 9 - protein, 120 aa, Mus musculus
EVTLVESGGGLVKPGGSLKLSCAASGFTFSTYVMSWVRQTPEKRLEWVASILSGGTSFYADNVKGRFTISRENARNILYLQMSSLKSEDTAMYYCVRRYGHDHYYAMDYWGQGTSVTVSS

SEQ ID NO: 10 - protein, 108 aa, Mus musculus
QIVLTQSPANMSASLGERVTMTCAASSSVSSSYLHWYQQKPGSSPKLWIYSTSNLASGVPGRFNGSGSGTSYSLTISSMEAEDAATYYCHQYHRSPWTFGGGTKLEIK

SEQ ID NO: 11 - DNA, 324 bp, Artificial Sequence
  Humanized antibody (T1L1)
gagatcgtgctgacacagtctcccgccacactgtcactgtctccaggcgaaagagccacactgagctgcgctgcctctagctctgtgtccagcagctacctgcactggtatcagcagaagcctggactggcccctcggctgctgatctacagcacaagcaatctggccagcggcatccccgatagattttccggctctggctccggcaccgacttcaccctgacaatcagcagactggaacccgaggacttcgccgtgtactactgccagcagtaccacagaagcccctggacatttggcggaggcaccaaggtggaaatcaag

SEQ ID NO: 12 - DNA, 324 bp, Artificial Sequence
  Humanized antibody (T1L2)
gagatcgtgctgacacagtctcccgccacactgtcactgtctccaggcgaaagagccacactgagctgcgctgcctctagctctgtgtccagcagctacctgcactggtatcagcagaagcctggcagcgctcccagactgctgatctacagcacaagcaatctggccagcggcatccccgatagattttccggctctggctccggcaccgacttcaccctgacaatcagcagactggaacccgaggacttcgccgtgtactactgccagcagtaccacagaagcccctggacatttggcggaggcaccaaggtggaaatcaag

SEQ ID NO: 13 - DNA, 324 bp, Artificial Sequence
  Humanized antibody (T1L3)
gagatcgtgctgacacagtctcccgccacactgtcactgtctccaggcgaaagagccacactgagctgcgctgcctctagctctgtgtccagcagctacctgcactggtatcagcagaagcctggcagcgctcccagactgctgatctacagcacaagcaatctggccagcggcatccccgatagattttccggctctggctccggcaccgacttcaccctgacaatctctagactggaagccgaggacttcgccgtgtactactgccagcagtaccacagaagcccctggacatttggcggaggcaccaaggtggaaatcaag

SEQ ID NO: 14 - DNA, 324 bp, Artificial Sequence
  Humanized antibody (T2L1)
gacatccagatgacacagagccccagcacactgtctgccagcgtgggagacagagtgaccattacatgtgccgccagcagcagcgtgtccagctcttacctgcactggtatcagcagaagcccggcaaggcccctaagctgctgatctacagcaccagcaatctggccagcggcgtgccaagcagattttctggctctggcagcggcaccgagttcaccctgaccatctctagcctgcagcctgacgacttcgccacctactactgccagcagtaccacagaagcccctggacatttggccagggcaccaagctggaaatcaag

SEQ ID NO: 15 - DNA, 324 bp, Artificial Sequence
  Humanized antibody (T2L2)
gacatccagatgacacagagccccagcacactgtctgccagcgtgggagacagagtgaccattacatgtgccgccagcagcagcgtgtccagctcttacctgcactggtatcagcagaagcccggcaaggcccctaagctgctgatctacagcaccagcaatctggccagcggcgtgccaagcagattttctggctctggcagcggcaccgagttcaccctgaccatctctagcctgcagcctgatgatgccgccacctactactgccagcagtaccacagaagcccctggacatttggccagggcaccaagctggaaatcaag

SEQ ID NO: 16 - DNA, 360 bp, Artificial Sequence
  Humanized antibody (T1H1)
gaggtgcagctggttgaatctggcggcggactgattcagcctggcggatctctgagactgagctgtgccgccagcggcttcacctttagcacctacgtgatgagctgggtccgacaggcccctggcaaaggacttgaatgggtgtccagcatcctgagcggcggcacaagcttctacgccgacaatgtgaagggcagattcaccatcagccgggacaacagcaagaacaccctgtacctgcagatgaacagcctgagagccgaggacaccgccgtgtactactgcgccagaagatacggccacgaccactactacgccatggactattggggccagggcaccctggttaccgttagctct

SEQ ID NO: 17 - DNA, 360 bp, Artificial Sequence
  Humanized antibody (T1H2)
gaggtgcagctggttgaatctggcggcggactgattcagcctggcggatctctgagactgagctgtgccgccagcggcttcacctttagcacctacgtgatgagctgggtccgacagacacctggcaaaggcctggaatgggtgtccagcattctgagcggcggcaccagcttctacgccgacaatgtgaagggcagattcaccatcagccgggacaacagcaagaacaccctgtacctgcagatgaacagcctgagagccgaggacaccgccgtgtactactgcgccagaagatacggccacgaccactactacgccatggactattggggccagggcaccctggttaccgttagctct

SEQ ID NO: 18 - DNA, 360 bp, Artificial Sequence
  Humanized antibody (T1H3)
gaggtgcagctggttgaatctggcggcggactgattcagcctggcggatctctgagactgagctgtgccgccagcggcttcacctttagcacctacgtgatgagctgggtccgacagacacctggcaaaggcctggaatgggtgtccagcattctgagcggcggcaccagcttctacgccgacaatgtgaagggcagattcaccatcagccgggacaacagcaagaacaccctgtacctgcagatgaacagcctgagagccgaggacaccgccatgtactactgcgccagaagatacggccacgaccactactacgccatggattattggggccagggcaccctggtcaccgtttcttct

SEQ ID NO: 19 - DNA, 360 bp, Artificial Sequence
  Humanized antibody (T2H1)
gaggtgcagctggttgaatctggtggcggcgttgtcagacctggcggatctctgagactgagctgtgccgccagcggcttcacctttagcacctacgtgatgagctgggtccgacaggcccctggcaaaggacttgaatgggtgtccagcatcctgagcggcggcacaagcttctacgccgacaatgtgaagggcagattcaccatcagccgggacaacgccaagaacagcctgtacctgcagatgaactccctgagagccgaggacacagccctgtatcactgcgccagaagatacggccacgaccactactacgccatggactattggggccagggcaccaccgtgacagtctcttct

SEQ ID NO: 20 - DNA, 360 bp, Artificial Sequence
  Humanized antibody (T2H2)
gaggtgcagctggttgaatctggtggcggcgttgtcagacctggcggatctctgagactgagctgtgccgccagcggcttcacctttagcacctacgtgatgagctgggtccgacagacacctggcaaaggcctggaatgggtgtccagcattctgagcggcggcaccagcttctacgccgacaatgtgaagggcagattcaccatcagccgggacaacgccaagaacagcctgtacctgcagatgaactccctgagagccgaggacacagccctgtatcactgcgccagaagatacggccacgaccactactacgccatggactattggggccagggcaccaccgtgacagtctcttct

SEQ ID NO: 21 - protein, 108 aa, Artificial Sequence
  Humanized antibody (T1L1)
EIVLTQSPATLSLSPGERATLSCAASSSVSSSYLHWYQQKPGLAPRLLIYSTSNLASGIPDRFSGSGSGTDFTLTISRLEPEDFAVYYCQQYHRSPWTFGGGTKVEIK

SEQ ID NO: 22 - protein, 108 aa, Artificial Sequence
  Humanized antibody (T1L2)
EIVLTQSPATLSLSPGERATLSCAASSSVSSSYLHWYQQKPGSAPRLLIYSTSNLASGIPDRFSGSGSGTDFTLTISRLEPEDFAVYYCQQYHRSPWTFGGGTKVEIK

SEQ ID NO: 23 - protein, 108 aa, Artificial Sequence
  Humanized antibody (T1L3)
EIVLTQSPATLSLSPGERATLSCAASSSVSSSYLHWYQQKPGSAPRLLIYSTSNLASGIPDRFSGSGSGTDFTLTISRLEAEDFAVYYCQQYHRSPWTFGGGTKVEIK

SEQ ID NO: 24 - protein, 108 aa, Artificial Sequence
  Humanized antibody (T2L1)
DIQMTQSPSTLSASVGDRVTITCAASSSVSSSYLHWYQQKPGKAPKLLIYSTSNLASGVPSRFSGSGSGTEFTLTISSLQPDDFATYYCQQYHRSPWTFGQGTKLEIK

SEQ ID NO: 25 - protein, 108 aa, Artificial Sequence
  Humanized antibody (T2L2)
DIQMTQSPSTLSASVGDRVTITCAASSSVSSSYLHWYQQKPGKAPKLLIYSTSNLASGVPSRFSGSGSGTEFTLTISSLQPDDAATYYCQQYHRSPWTFGQGTKLEIK

SEQ ID NO: 26 - protein, 120 aa, Artificial Sequence
  Humanized antibody (T1H1)
EVQLVESGGGLIQPGGSLRLSCAASGFTFSTYVMSWVRQAPGKGLEWVSSILSGGTSFYADNVKGRFTISRDNSKNTLYLQMNSLRAEDTAVYYCARRYGHDHYYAMDYWGQGTLVTVSS

SEQ ID NO: 27 - protein, 120 aa, Artificial Sequence
  Humanized antibody (T1H2)
EVQLVESGGGLIQPGGSLRLSCAASGFTFSTYVMSWVRQTPGKGLEWVSSILSGGTSFYADNVKGRFTISRDNSKNTLYLQMNSLRAEDTAVYYCARRYGHDHYYAMDYWGQGTLVTVSS

SEQ ID NO: 28 - protein, 120 aa, Artificial Sequence
  Humanized antibody (T1H3)
EVQLVESGGGLIQPGGSLRLSCAASGFTFSTYVMSWVRQTPGKGLEWVSSILSGGTSFYADNVKGRFTISRDNSKNTLYLQMNSLRAEDTAMYYCARRYGHDHYYAMDYWGQGTLVTVSS

SEQ ID NO: 29 - protein, 120 aa, Artificial Sequence
  Humanized antibody (T2H1)
EVQLVESGGGVVRPGGSLRLSCAASGFTFSTYVMSWVRQAPGKGLEWVSSILSGGTSFYADNVKGRFTISRDNAKNSLYLQMNSLRAEDTALYHCARRYGHDHYYAMDYWGQGTTVTVSS

SEQ ID NO: 30 - protein, 120 aa, Artificial Sequence
  Humanized antibody (T2H2)
EVQLVESGGGVVRPGGSLRLSCAASGFTFSTYVMSWVRQTPGKGLEWVSSILSGGTSFYADNVKGRFTISRDNAKNSLYLQMNSLRAEDTALYHCARRYGHDHYYAMDYWGQGTTVTVSS

SEQ ID NO: 31 - protein, 20 aa, Artificial Sequence
  IL-2 signal peptide
MYRMQLLSCIALSLALVTNS

SEQ ID NO: 32 - protein, 288 aa, Artificial Sequence
  CD276 Fragment
LEVQVPEDPVVALVGTDATLCCSFSPEPGFSLAQLNLIWQLTDTKQLVHSFAEGQDQGSAYANRTALFPDLLAQGNASLRLQRVRVADEGSFTCFVSIRDFGSAAVSLQVAAPYSKPSMTLEPNKDLRPGDTVTITCSSYRGYPEAEVFWQDGQGVPLTGNVTTSQMANEQGLFDVHSVLRVVLGANGTYSCLVRNPVLQQDAHGSVTITGQPMTFPPEALWVTVGLSVCLIALLVALAFVCWRKIKQSCEEENAGAEDQDGEGEGSKTALQPLKHSDSKEDDGQEIA

SEQ ID NO: 33 - protein, 316 aa, Artificial Sequence
  CD276 Fragment
MLRRRGSPGMGVHVGAALGALWFCLTGALEVQVPEDPVVALVGTDATLCCSFSPEPGFSLAQLNLIWQLTDTKQLVHSFAEGQDQGSAYANRTALFPDLLAQGNASLRLQRVRVADEGSFTCFVSIRDFGSAAVSLQVAAPYSKPSMTLEPNKDLRPGDTVTITCSSYRGYPEAEVFWQDGQGVPLTGNVTTSQMANEQGLFDVHSVLRVVLGANGTYSCLVRNPVLQQDAHGSVTITGQPMTFPPEALWVTVGLSVCLIALLVALAFVCWRKIKQSCEEENAGAEDQDGEGEGSKTALQPLKHSDSKEDDGQEIA